European Patent Application EP 4 454 710 A1, published October 30, 2024. Title: Bispecific fusion proteins with immunosuppressive activity. Applicant: UNIVERSITAT DE BARCELONA. The sequence listing filed with the application follows.

SEQUENCE LISTING (14 sequences)

SEQ ID NO: 1 - protein, 124 aa, Homo sapiens [sequence omitted]

SEQ ID NO: 2 - protein, 200 aa, Homo sapiens
FTVTVPKELYIIEHGSNVTLECNFDTGSHVNLGAITASLQKVENDTSPHRERATLLEEQLPLGKASFHIPQVQVRDEGQYQCIIIYGVAWDYKYLTLKVKASYRKINTHILKVPETDEVELTCQATGYPLAEVSWPNVSVPANTSHSRTPEGLYQVTSVLRLKPPPGRNFSCVFWNTHVRELTLASIDLQSQMEPRTHPT

SEQ ID NO: 3 - protein, 233 aa, Homo sapiens
QEPKSSDKTHTSPPSPAPELLGGSSVFLFPPKPKDTLMISRTPEVTCVVVDVSHEDPEVKFNWYVDGVEVHNAKTKPREEQYNSTYRVVSVLTVLHQDWLNGKEYKCKVSNKALPAPIEKTISKAKGQPREPQVYTLPPSRDELTKNQVSLTCLVKGFYPSDIAVEWESNGQPENNYKTTPPVLDSDGSFFLYSKLTVDKSRWQQGNVFSCSVMHEALHNHYTQKSLSLSPGK

SEQ ID NO: 4 - protein, 12 aa, synthetic construct
  VARIANT 1..2: note = X represents E or D
  VARIANT 7..8: note = X represents E or D
  REGION >1: note = The entire sequence of amino acids 1 to 12 can be repeated from 2 to 10 times
XXAAKKXXAAKK

SEQ ID NO: 5 - protein, 8 aa, synthetic construct
  VARIANT 1..8: note = X represents an acidic or basic amino acid
  REGION >8: note = The amino acids at positions 1-2 can be repeated from 2 to 20 times
XPXPXPXP

SEQ ID NO: 6 - protein, 8 aa, synthetic construct
  VARIANT 1..8: note = X represents an acidic or basic amino acid
  REGION >1: note = The amino acids at positions 1-2 can be repeated from 2 to 20 times
PXPXPXPX

SEQ ID NO: 7 - protein, 28 aa, synthetic construct
  VARIANT 1..28: note = X represents an acidic or a basic amino acid
  REGION >1: note = The entire sequence can be repeated from 2 to 20 times
XPXPXPXPXPXPGGXPXPXPXPXPXPGG

SEQ ID NO: 8 - protein, 5 aa, synthetic construct
EAAAK

SEQ ID NO: 9 - protein, 17 aa, synthetic construct
  REGION >2: note = The sequence of amino acids at positions 2 to 6 are repeated up to 8 times
AEAAAKEAAAKEAAAKA

SEQ ID NO: 10 - protein, 32 aa, synthetic construct
AEAAAKEAAAKEAAAKEAAAKEAAAKEAAAKA

SEQ ID NO: 11 - protein, 589 aa, synthetic construct
  REGION 1..589: note = Fusion polypeptide of formula I
MHVAQPAVVLASSRGIASFVCEYASPGKATEVRVTVLRQADSQVTEVCAATYMMGNELTFLDDSICTGTSSGNQVNLTIQGLRAMDTGLYICKVELMYPPPYYLGIGNGTQIYVIDPEPCPDSDQEPKSSDKTHTSPPSPAPELLGGSSVFLFPPKPKDTLMISRTPEVTCVVVDVSHEDPEVKFNWYVDGVEVHNAKTKPREEQYNSTYRVVSVLTVLHQDWLNGKEYKCKVSNKALPAPIEKTISKAKGQPREPQVYTLPPSRDELTKNQVSLTCLVKGFYPSDIAVEWESNGQPENNYKTTPPVLDSDGSFFLYSKLTVDKSRWQQGNVFSCSVMHEALHNHYTQKSLSLSPGKAEAAAKEAAAKEAAAKEAAAKEAAAKEAAAKAFTVTVPKELYIIEHGSNVTLECNFDTGSHVNLGAITASLQKVENDTSPHRERATLLEEQLPLGKASFHIPQVQVRDEGQYQCIIIYGVAWDYKYLTLKVKASYRKINTHILKVPETDEVELTCQATGYPLAEVSWPNVSVPANTSHSRTPEGLYQVTSVLRLKPPPGRNFSCVFWNTHVRELTLASIDLQSQMEPRTHPT

SEQ ID NO: 12 - DNA, 1881 bp, synthetic construct
  source 1..1881: mol_type = other DNA
atggcctgcctgggcttccagaggcacaaggcccagctgaacctggctacccggacatggccttgcaccctgctgttctttctgctgttcatcccagtgttttgtaaggctatgcatgtggctcagccagctgtggtgctggcctccagcaggggaatcgcctccttcgtgtgcgagtacgcctctcccggcaaggctaccgaggtgagagtgacagtgctgaggcaggctgacagccaggtgaccgaggtgtgcgccgctacatatatgatgggcaacgagctgacctttctggacgattctatctgtaccggcacatcttccggcaaccaagtgaatctgaccatccagggcctgcgggctatggatacaggcctgtacatctgcaaggtggagctgatgtatccccctccatactatctgggcatcggcaatggcacccagatctacgtgatcgacccagagccctgtcctgactctgatcaggagcctaagagctctgataagacccacacatccccacctagcccagctccagagctgctgggcggctccagcgtgttcctgtttccacccaagccaaaggacaccctgatgatcagcagaacccccgaggtgacatgcgtggtggtggacgtgtctcacgaggatccagaggtgaagtttaactggtacgtggatggcgtggaggtgcataatgccaagacaaagcccagagaggagcagtacaattctacctatcgcgtggtgtccgtgctgacagtgctgcatcaggactggctgaacggcaaggagtataagtgcaaggtgtccaataaggccctgcctgctccaatcgagaagaccatcagcaaggccaagggccagcccagagagcctcaggtgtacacactgcctccatcccgcgacgagctgaccaagaaccaggtgagcctgacatgtctggtgaagggcttctatccttctgatatcgctgtggagtgggagtccaatggccagccagagaacaattacaagaccacaccccctgtgctggactctgatggctccttctttctgtattccaagctgaccgtggataagagccgctggcagcagggcaacgtgttttcttgctccgtgatgcacgaggccctgcacaatcattacacacagaagagcctgtctctgtcccctggcaaggctgaggctgctgctaaggaagccgctgctaaggaggccgctgccaaggaggctgccgctaaggaggctgctgccaaagaggctgctgctaaggccttcaccgtgacagtgccaaaggagctgtatatcatcgagcacggctctaacgtgaccctggagtgtaattttgacacaggctcccatgtgaacctgggcgccatcaccgcctccctgcagaaggtggagaatgatacctctccacacagggagagggccacactgctggaggagcagctgccactgggcaaggcttccttccatatccctcaggtgcaggtgagagacgagggccagtaccagtgcatcatcatctatggcgtggcctgggattacaagtatctgaccctgaaggtgaaggcctcctaccgcaagatcaacacccacatcctgaaggtgcccgagacagacgaggtggagctgacctgtcaggccacaggctatcctctggctgaggtgagctggcctaacgtgtctgtgccagccaataccagccattctagaacacctgagggcctgtaccaggtgacctctgtgctgaggctgaagccaccacctggaaggaacttctcctgcgtgttctggaatacccacgtgagggagctgacactggcttccatcgatctgcagagccagatggagccacggacccatcccacatga

SEQ ID NO: 13 - DNA, 7299 bp, synthetic construct
  source 1..7299: mol_type = other DNA
gacggatcgggagatctcccgatcccctatggtgcactctcagtacaatctgctctgatgccgcatagttaagccagtatctgctccctgcttgtgtgttggaggtcgctgagtagtgcgcgagcaaaatttaagctacaacaaggcaaggcttgaccgacaattgcatgaagaatctgcttagggttaggcgttttgcgctgcttcgcgatgtacgggccagatatacgcgttgacattgattattgactagttattaatagtaatcaattacggggtcattagttcatagcccatatatggagttccgcgttacataacttacggtaaatggcccgcctggctgaccgcccaacgacccccgcccattgacgtcaataatgacgtatgttcccatagtaacgccaatagggactttccattgacgtcaatgggtggagtatttacggtaaactgcccacttggcagtacatcaagtgtatcatatgccaagtacgccccctattgacgtcaatgacggtaaatggcccgcctggcattatgcccagtacatgaccttatgggactttcctacttggcagtacatctacgtattagtcatcgctattaccatggtgatgcggttttggcagtacatcaatgggcgtggatagcggtttgactcacggggatttccaagtctccaccccattgacgtcaatgggagtttgttttggcaccaaaatcaacgggactttccaaaatgtcgtaacaactccgccccattgacgcaaatgggcggtaggcgtgtacggtgggaggtctatataagcagagctctctggctaactagagaacccactgcttactggcttatcgaaattaatacgactcactatagggagacccaagctggctagcatggcctgcctgggcttccagaggcacaaggcccagctgaacctggctacccggacatggccttgcaccctgctgttctttctgctgttcatcccagtgttttgtaaggctatgcatgtggctcagccagctgtggtgctggcctccagcaggggaatcgcctccttcgtgtgcgagtacgcctctcccggcaaggctaccgaggtgagagtgacagtgctgaggcaggctgacagccaggtgaccgaggtgtgcgccgctacatatatgatgggcaacgagctgacctttctggacgattctatctgtaccggcacatcttccggcaaccaagtgaatctgaccatccagggcctgcgggctatggatacaggcctgtacatctgcaaggtggagctgatgtatccccctccatactatctgggcatcggcaatggcacccagatctacgtgatcgacccagagccctgtcctgactctgatcaggagcctaagagctctgataagacccacacatccccacctagcccagctccagagctgctgggcggctccagcgtgttcctgtttccacccaagccaaaggacaccctgatgatcagcagaacccccgaggtgacatgcgtggtggtggacgtgtctcacgaggatccagaggtgaagtttaactggtacgtggatggcgtggaggtgcataatgccaagacaaagcccagagaggagcagtacaattctacctatcgcgtggtgtccgtgctgacagtgctgcatcaggactggctgaacggcaaggagtataagtgcaaggtgtccaataaggccctgcctgctccaatcgagaagaccatcagcaaggccaagggccagcccagagagcctcaggtgtacacactgcctccatcccgcgacgagctgaccaagaaccaggtgagcctgacatgtctggtgaagggcttctatccttctgatatcgctgtggagtgggagtccaatggccagccagagaacaattacaagaccacaccccctgtgctggactctgatggctccttctttctgtattccaagctgaccgtggataagagccgctggcagcagggcaacgtgttttcttgctccgtgatgcacgaggccctgcacaatcattacacacagaagagcctgtctctgtcccctggcaaggctgaggctgctgctaaggaagccgctgctaaggaggccgctgccaaggaggctgccgctaaggaggctgctgccaaagaggctgctgctaaggccttcaccgtgacagtgccaaaggagctgtatatcatcgagcacggctctaacgtgaccctggagtgtaattttgacacaggctcccatgtgaacctgggcgccatcaccgcctccctgcagaaggtggagaatgatacctctccacacagggagagggccacactgctggaggagcagctgccactgggcaaggcttccttccatatccctcaggtgcaggtgagagacgagggccagtaccagtgcatcatcatctatggcgtggcctgggattacaagtatctgaccctgaaggtgaaggcctcctaccgcaagatcaacacccacatcctgaaggtgcccgagacagacgaggtggagctgacctgtcaggccacaggctatcctctggctgaggtgagctggcctaacgtgtctgtgccagccaataccagccattctagaacacctgagggcctgtaccaggtgacctctgtgctgaggctgaagccaccacctggaaggaacttctcctgcgtgttctggaatacccacgtgagggagctgacactggcttccatcgatctgcagagccagatggagccacggacccatcccacatgataaggtaccgagctcggatccactagtccagtgtggtggaattctgcagatatccagcacagtggcggccgctcgagtctagagggcccgtttaaacccgctgatcagcctcgactgtgccttctagttgccagccatctgttgtttgcccctcccccgtgccttccttgaccctggaaggtgccactcccactgtcctttcctaataaaatgaggaaattgcatcgcattgtctgagtaggtgtcattctattctggggggtggggtggggcaggacagcaagggggaggattgggaagacaatagcaggcatgctggggatgcggtgggctctatggcttctgaggcggaaagaaccagctggggctctagggggtatccccacgcgccctgtagcggcgcattaagcgcggcgggtgtggtggttacgcgcagcgtgaccgctacacttgccagcgccctagcgcccgctcctttcgctttcttcccttcctttctcgccacgttcgccggctttccccgtcaagctctaaatcgggggctccctttagggttccgatttagtgctttacggcacctcgaccccaaaaaacttgattagggtgatggttcacgtagtgggccatcgccctgatagacggtttttcgccctttgacgttggagtccacgttctttaatagtggactcttgttccaaactggaacaacactcaaccctatctcggtctattcttttgatttataagggattttgccgatttcggcctattggttaaaaaatgagctgatttaacaaaaatttaacgcgaattaattctgtggaatgtgtgtcagttagggtgtggaaagtccccaggctccccagcaggcagaagtatgcaaagcatgcatctcaattagtcagcaaccaggtgtggaaagtccccaggctccccagcaggcagaagtatgcaaagcatgcatctcaattagtcagcaaccatagtcccgcccctaactccgcccatcccgcccctaactccgcccagttccgcccattctccgccccatggctgactaattttttttatttatgcagaggccgaggccgcctctgcctctgagctattccagaagtagtgaggaggcttttttggaggcctaggcttttgcaaaaagctcccgggagcttgtatatccattttcggatctgatcaagagacaggatgaggatcgtttcgcatgattgaacaagatggattgcacgcaggttctccggccgcttgggtggagaggctattcggctatgactgggcacaacagacaatcggctgctctgatgccgccgtgttccggctgtcagcgcaggggcgcccggttctttttgtcaagaccgacctgtccggtgccctgaatgaactgcaggacgaggcagcgcggctatcgtggctggccacgacgggcgttccttgcgcagctgtgctcgacgttgtcactgaagcgggaagggactggctgctattgggcgaagtgccggggcaggatctcctgtcatctcaccttgctcctgccgagaaagtatccatcatggctgatgcaatgcggcggctgcatacgcttgatccggctacctgcccattcgaccaccaagcgaaacatcgcatcgagcgagcacgtactcggatggaagccggtcttgtcgatcaggatgatctggacgaagagcatcaggggctcgcgccagccgaactgttcgccaggctcaaggcgcgcatgcccgacggcgaggatctcgtcgtgacccatggcgatgcctgcttgccgaatatcatggtggaaaatggccgcttttctggattcatcgactgtggccggctgggtgtggcggaccgctatcaggacatagcgttggctacccgtgatattgctgaagagcttggcggcgaatgggctgaccgcttcctcgtgctttacggtatcgccgctcccgattcgcagcgcatcgccttctatcgccttcttgacgagttcttctgagcgggactctggggttcgaaatgaccgaccaagcgacgcccaacctgccatcacgagatttcgattccaccgccgccttctatgaaaggttgggcttcggaatcgttttccgggacgccggctggatgatcctccagcgcggggatctcatgctggagttcttcgcccaccccaacttgtttattgcagcttataatggttacaaataaagcaatagcatcacaaatttcacaaataaagcatttttttcactgcattctagttgtggtttgtccaaactcatcaatgtatcttatcatgtctgtataccgtcgacctctagctagagcttggcgtaatcatggtcatagctgtttcctgtgtgaaattgttatccgctcacaattccacacaacatacgagccggaagcataaagtgtaaagcctggggtgcctaatgagtgagctaactcacattaattgcgttgcgctcactgcccgctttccagtcgggaaacctgtcgtgccagctgcattaatgaatcggccaacgcgcggggagaggcggtttgcgtattgggcgctcttccgcttcctcgctcactgactcgctgcgctcggtcgttcggctgcggcgagcggtatcagctcactcaaaggcggtaatacggttatccacagaatcaggggataacgcaggaaagaacatgtgagcaaaaggccagcaaaaggccaggaaccgtaaaaaggccgcgttgctggcgtttttccataggctccgcccccctgacgagcatcacaaaaatcgacgctcaagtcagaggtggcgaaacccgacaggactataaagataccaggcgtttccccctggaagctccctcgtgcgctctcctgttccgaccctgccgcttaccggatacctgtccgcctttctcccttcgggaagcgtggcgctttctcatagctcacgctgtaggtatctcagttcggtgtaggtcgttcgctccaagctgggctgtgtgcacgaaccccccgttcagcccgaccgctgcgccttatccggtaactatcgtcttgagtccaacccggtaagacacgacttatcgccactggcagcagccactggtaacaggattagcagagcgaggtatgtaggcggtgctacagagttcttgaagtggtggcctaactacggctacactagaagaacagtatttggtatctgcgctctgctgaagccagttaccttcggaaaaagagttggtagctcttgatccggcaaacaaaccaccgctggtagcggtggtttttttgtttgcaagcagcagattacgcgcagaaaaaaaggatctcaagaagatcctttgatcttttctacggggtctgacgctcagtggaacgaaaactcacgttaagggattttggtcatgagattatcaaaaaggatcttcacctagatccttttaaattaaaaatgaagttttaaatcaatctaaagtatatatgagtaaacttggtctgacagttaccaatgcttaatcagtgaggcacctatctcagcgatctgtctatttcgttcatccatagttgcctgactccccgtcgtgtagataactacgatacgggagggcttaccatctggccccagtgctgcaatgataccgcgagacccacgctcaccggctccagatttatcagcaataaaccagccagccggaagggccgagcgcagaagtggtcctgcaactttatccgcctccatccagtctattaattgttgccgggaagctagagtaagtagttcgccagttaatagtttgcgcaacgttgttgccattgctacaggcatcgtggtgtcacgctcgtcgtttggtatggcttcattcagctccggttcccaacgatcaaggcgagttacatgatcccccatgttgtgcaaaaaagcggttagctccttcggtcctccgatcgttgtcagaagtaagttggccgcagtgttatcactcatggttatggcagcactgcataattctcttactgtcatgccatccgtaagatgcttttctgtgactggtgagtactcaaccaagtcattctgagaatagtgtatgcggcgaccgagttgctcttgcccggcgtcaatacgggataataccgcgccacatagcagaactttaaaagtgctcatcattggaaaacgttcttcggggcgaaaactctcaaggatcttaccgctgttgagatccagttcgatgtaacccactcgtgcacccaactgatcttcagcatcttttactttcaccagcgtttctgggtgagcaaaaacaggaaggcaaaatgccgcaaaaaagggaataagggcgacacggaaatgttgaatactcatactcttcctttttcaatattattgaagcatttatcagggttattgtctcatgagcggatacatatttgaatgtatttagaaaaataaacaaataggggttccgcgcacatttccccgaaaagtgccacctgacgtc

SEQ ID NO: 14 - protein, 626 aa, synthetic construct
  REGION 1..626: note = Fusion polypeptide of formula I including at the N-terminal a signal peptide
MACLGFQRHKAQLNLATRTWPCTLLFFLLFIPVFCKAMHVAQPAVVLASSRGIASFVCEYASPGKATEVRVTVLRQADSQVTEVCAATYMMGNELTFLDDSICTGTSSGNQVNLTIQGLRAMDTGLYICKVELMYPPPYYLGIGNGTQIYVIDPEPCPDSDQEPKSSDKTHTSPPSPAPELLGGSSVFLFPPKPKDTLMISRTPEVTCVVVDVSHEDPEVKFNWYVDGVEVHNAKTKPREEQYNSTYRVVSVLTVLHQDWLNGKEYKCKVSNKALPAPIEKTISKAKGQPREPQVYTLPPSRDELTKNQVSLTCLVKGFYPSDIAVEWESNGQPENNYKTTPPVLDSDGSFFLYSKLTVDKSRWQQGNVFSCSVMHEALHNHYTQKSLSLSPGKAEAAAKEAAAKEAAAKEAAAKEAAAKEAAAKAFTVTVPKELYIIEHGSNVTLECNFDTGSHVNLGAITASLQKVENDTSPHRERATLLEEQLPLGKASFHIPQVQVRDEGQYQCIIIYGVAWDYKYLTLKVKASYRKINTHILKVPETDEVELTCQATGYPLAEVSWPNVSVPANTSHSRTPEGLYQVTSVLRLKPPPGRNFSCVFWNTHVRELTLASIDLQSQMEPRTHPT